European Patent Application EP 4 512 886 A1, published February 26, 2025. Title: 核酸检测装置及核酸检测方法. Applicant: 长庚大学. Application CN. The sequence listing filed with the application follows.

SEQUENCE LISTING (3 sequences)

SEQ ID NO: 1 - DNA, 188 bp, Agrobacterium tumefaciens
  source 1..188: mol_type = other DNA; organism (original language) = 根癌农杆菌
ttgaggagacggataaagttgttgcactcgagctaggagcaagtgattttatcgctaagccgtttagtacgagagagtttcttgcacgcattcgggttgccttgcgcgtgcgccccaacgttgtccgctccaaagaccgacggtctttttgttttactgactggacacttaatctcaggcaacgtcgc

SEQ ID NO: 2 - DNA, 30 bp, synthetic construct
  source 1..30: mol_type = other DNA; organism (original language) = 合成结构
ttgaggagacggataaagttgttgcactcg

SEQ ID NO: 3 - DNA, 30 bp, synthetic construct
  source 1..30: mol_type = other DNA; organism (original language) = 合成结构
gcgacgttgcctgagattaagtgtccagtc